European Patent Application EP 4 768 032 A1, published July 1, 2026. Title: 靶向RAGE的RNAi剂及其医药用途. Applicant: 上海拓界生物医药科技有限公司. Application WO. The sequence listing filed with the application follows.

SEQUENCE LISTING (278 sequences)

SEQ ID NO: 1 - RNA, 19 nt, Homo sapiens
  source 1..19: mol_type = mRNA
ctgtcagcatcagcatcaa

SEQ ID NO: 2 - RNA, 19 nt, Homo sapiens
  source 1..19: mol_type = mRNA
gaccaactctctcctgtaa

SEQ ID NO: 3 - RNA, 19 nt, Homo sapiens
  source 1..19: mol_type = mRNA
agaggaggagcgtgcagaa

SEQ ID NO: 4 - RNA, 19 nt, Homo sapiens
  source 1..19: mol_type = mRNA
cagtcggagctaatggtga

SEQ ID NO: 5 - RNA, 19 nt, Homo sapiens
  source 1..19: mol_type = mRNA
cttttctttttcccttgaa

SEQ ID NO: 6 - RNA, 19 nt, Homo sapiens
  source 1..19: mol_type = mRNA
ccttttctttttcccttga

SEQ ID NO: 7 - RNA, 19 nt, Homo sapiens
  source 1..19: mol_type = mRNA
ctgtcagcatcagcatcat

SEQ ID NO: 8 - RNA, 19 nt, Homo sapiens
  source 1..19: mol_type = mRNA
gaccaactctctcctgtat

SEQ ID NO: 9 - RNA, 19 nt, synthetic construct
  source 1..19: mol_type = other RNA; note; note (original language) = 第7-9位为2'-氟代修饰；其余位置为2'-甲氧基修饰。硫代磷酸二酯基位于5'端第1和第2核苷酸、第2和第3核苷酸之间。
ctgtcagcatcagcatcaa

SEQ ID NO: 10 - RNA, 19 nt, synthetic construct
  source 1..19: mol_type = other RNA; note; note (original language) = 第7-9位为2'-氟代修饰；其余位置为2'-甲氧基修饰。硫代磷酸二酯基位于5'端第1和第2核苷酸、第2和第3核苷酸之间。
gaccaactctctcctgtaa

SEQ ID NO: 11 - RNA, 19 nt, synthetic construct
  source 1..19: mol_type = other RNA; note; note (original language) = 第7-9位为2'-氟代修饰；其余位置为2'-甲氧基修饰。硫代磷酸二酯基位于5'端第1和第2核苷酸、第2和第3核苷酸之间。
agaggaggagcgtgcagaa

SEQ ID NO: 12 - RNA, 19 nt, synthetic construct
  source 1..19: mol_type = other RNA; note; note (original language) = 第7-9位为2'-氟代修饰；其余位置为2'-甲氧基修饰。硫代磷酸二酯基位于5'端第1和第2核苷酸、第2和第3核苷酸之间。
cagtcggagctaatggtga

SEQ ID NO: 13 - RNA, 19 nt, synthetic construct
  source 1..19: mol_type = other RNA; note; note (original language) = 第7-9位为2'-氟代修饰；其余位置为2'-甲氧基修饰。硫代磷酸二酯基位于5'端第1和第2核苷酸、第2和第3核苷酸之间。
cttttctttttcccttgaa

SEQ ID NO: 14 - RNA, 19 nt, synthetic construct
  source 1..19: mol_type = other RNA; note; note (original language) = 第7-9位为2'-氟代修饰；其余位置为2'-甲氧基修饰。硫代磷酸二酯基位于5'端第1和第2核苷酸、第2和第3核苷酸之间。
ccttttctttttcccttga

SEQ ID NO: 15 - RNA, 19 nt, synthetic construct
  source 1..19: mol_type = other RNA; note; note (original language) = 第7-9位为2'-氟代修饰；其余位置为2'-甲氧基修饰。硫代磷酸二酯基位于5'端第1和第2核苷酸、第2和第3核苷酸之间；3'端第1和第2核苷酸、第2和第3核苷酸之间。
ctgtcagcatcagcatcaa

SEQ ID NO: 16 - RNA, 19 nt, synthetic construct
  source 1..19: mol_type = other RNA; note; note (original language) = 第7-9位为2'-氟代修饰；其余位置为2'-甲氧基修饰。硫代磷酸二酯基位于5'端第1和第2核苷酸、第2和第3核苷酸之间；3'端第1和第2核苷酸、第2和第3核苷酸之间。
gaccaactctctcctgtaa

SEQ ID NO: 17 - RNA, 19 nt, synthetic construct
  source 1..19: mol_type = other RNA; note; note (original language) = 第7-9位为2'-氟代修饰；其余位置为2'-甲氧基修饰。硫代磷酸二酯基位于5'端第1和第2核苷酸、第2和第3核苷酸之间；3'端第1和第2核苷酸、第2和第3核苷酸之间。
agaggaggagcgtgcagaa

SEQ ID NO: 18 - RNA, 19 nt, synthetic construct
  source 1..19: mol_type = other RNA; note; note (original language) = 第7-9位为2'-氟代修饰；其余位置为2'-甲氧基修饰。硫代磷酸二酯基位于5'端第1和第2核苷酸、第2和第3核苷酸之间；3'端第1和第2核苷酸、第2和第3核苷酸之间。
cagtcggagctaatggtga

SEQ ID NO: 19 - RNA, 19 nt, synthetic construct
  source 1..19: mol_type = other RNA; note; note (original language) = 第7-9位为2'-氟代修饰；其余位置为2'-甲氧基修饰。硫代磷酸二酯基位于5'端第1和第2核苷酸、第2和第3核苷酸之间；3'端第1和第2核苷酸、第2和第3核苷酸之间。
cttttctttttcccttgaa

SEQ ID NO: 20 - RNA, 19 nt, synthetic construct
  source 1..19: mol_type = other RNA; note; note (original language) = 第7-9位为2'-氟代修饰；其余位置为2'-甲氧基修饰。硫代磷酸二酯基位于5'端第1和第2核苷酸、第2和第3核苷酸之间；3'端第1和第2核苷酸、第2和第3核苷酸之间。
ccttttctttttcccttga

SEQ ID NO: 21 - RNA, 19 nt, synthetic construct
  source 1..19: mol_type = other RNA; note; note (original language) = 第7-9位为2'-氟代修饰；其余位置为2'-甲氧基修饰。硫代磷酸二酯基位于5'端第1和第2核苷酸、第2和第3核苷酸之间；3'端第1和第2核苷酸、第2和第3核苷酸之间。5'端带有I-14配体。
ctgtcagcatcagcatcaa

SEQ ID NO: 22 - RNA, 19 nt, synthetic construct
  source 1..19: mol_type = other RNA; note; note (original language) = 第2、4、6、10、12、14、16、18位为2'-氟代修饰；其余位置为2'-甲氧基修饰。硫代磷酸二酯基位于5'端第1和第2核苷酸、第2和第3核苷酸之间；3'端第1和第2核苷酸、第2和第3
gaccaactctctcctgtaa

SEQ ID NO: 23 - RNA, 19 nt, synthetic construct
  source 1..19: mol_type = other RNA; note; note (original language) = 第7-9位为2'-氟代修饰；其余位置为2'-甲氧基修饰。硫代磷酸二酯基位于5'端第1和第2核苷酸、第2和第3核苷酸之间；3'端第1和第2核苷酸、第2和第3核苷酸之间。5'端带有I-14配体。
agaggaggagcgtgcagaa

SEQ ID NO: 24 - RNA, 19 nt, synthetic construct
  source 1..19: mol_type = other RNA; note; note (original language) = 第7-9位为2'-氟代修饰；其余位置为2'-甲氧基修饰。硫代磷酸二酯基位于5'端第1和第2核苷酸、第2和第3核苷酸之间；3'端第1和第2核苷酸、第2和第3核苷酸之间。5'端带有I-14配体。
cagtcggagctaatggtga

SEQ ID NO: 25 - RNA, 19 nt, synthetic construct
  source 1..19: mol_type = other RNA; note; note (original language) = 第7-9位为2'-氟代修饰；其余位置为2'-甲氧基修饰。硫代磷酸二酯基位于5'端第1和第2核苷酸、第2和第3核苷酸之间；3'端第1和第2核苷酸、第2和第3核苷酸之间。5'端带有I-14配体。
cttttctttttcccttgaa

SEQ ID NO: 26 - RNA, 19 nt, synthetic construct
  source 1..19: mol_type = other RNA; note; note (original language) = 第7-9位为2'-氟代修饰；其余位置为2'-甲氧基修饰。硫代磷酸二酯基位于5'端第1和第2核苷酸、第2和第3核苷酸之间；3'端第1和第2核苷酸、第2和第3核苷酸之间。5'端带有I-14配体。
ccttttctttttcccttga

SEQ ID NO: 27 - RNA, 21 nt, Homo sapiens
  source 1..21: mol_type = mRNA
ttgatgctgatgctgacagca

SEQ ID NO: 28 - RNA, 21 nt, Homo sapiens
  source 1..21: mol_type = mRNA
ttacaggagagagttggtctg

SEQ ID NO: 29 - RNA, 21 nt, Homo sapiens
  source 1..21: mol_type = mRNA
ttctgcacgctcctcctcttc

SEQ ID NO: 30 - RNA, 21 nt, Homo sapiens
  source 1..21: mol_type = mRNA
tcaccattagctccgactgca

SEQ ID NO: 31 - RNA, 21 nt, Homo sapiens
  source 1..21: mol_type = mRNA
ttcaagggaaaaagaaaaggg

SEQ ID NO: 32 - RNA, 21 nt, Homo sapiens
  source 1..21: mol_type = mRNA
tcaagggaaaaagaaaaggga

SEQ ID NO: 33 - RNA, 21 nt, Homo sapiens
  source 1..21: mol_type = mRNA
atgatgctgatgctgacagca

SEQ ID NO: 34 - RNA, 21 nt, Homo sapiens
  source 1..21: mol_type = mRNA
atacaggagagagttggtctg

SEQ ID NO: 35 - RNA, 21 nt, synthetic construct
  source 1..21: mol_type = other RNA; note; note (original language) = 5'端带有乙烯基磷酸二酯基。第2、6、12、14、16位为2'-氟代修饰；其余位置为2'-甲氧基修饰。硫代磷酸二酯基位于5'端第1和第2核苷酸、第2和第3核苷酸之间；3'端第1和第2核苷酸、第2和第3个苷酸之间。
ttgatgctgatgctgacagca

SEQ ID NO: 36 - RNA, 21 nt, synthetic construct
  source 1..21: mol_type = other RNA; note; note (original language) = 5'端带有乙烯基磷酸二酯基。第2、6、12、14、16位为2'-氟代修饰；其余位置为2'-甲氧基修饰。硫代磷酸二酯基位于5'端第1和第2核苷酸、第2和第3核苷酸之间；3'端第1和第2核苷酸、第2和第3个苷酸之间。
ttacaggagagagttggtctg

SEQ ID NO: 37 - RNA, 21 nt, synthetic construct
  source 1..21: mol_type = other RNA; note; note (original language) = 5'端带有乙烯基磷酸二酯基。第2、6、12、14、16位为2'-氟代修饰；其余位置为2'-甲氧基修饰。硫代磷酸二酯基位于5'端第1和第2核苷酸、第2和第3核苷酸之间；3'端第1和第2核苷酸、第2和第3个苷酸之间。
ttctgcacgctcctcctcttc

SEQ ID NO: 38 - RNA, 21 nt, synthetic construct
  source 1..21: mol_type = other RNA; note; note (original language) = 5'端带有乙烯基磷酸二酯基。第2、6、12、14、16位为2'-氟代修饰；其余位置为2'-甲氧基修饰。硫代磷酸二酯基位于5'端第1和第2核苷酸、第2和第3核苷酸之间；3'端第1和第2核苷酸、第2和第3个苷酸之间。
tcaccattagctccgactgca

SEQ ID NO: 39 - RNA, 21 nt, synthetic construct
  source 1..21: mol_type = other RNA; note; note (original language) = 5'端带有乙烯基磷酸二酯基。第2、6、12、14、16位为2'-氟代修饰；其余位置为2'-甲氧基修饰。硫代磷酸二酯基位于5'端第1和第2核苷酸、第2和第3核苷酸之间；3'端第1和第2核苷酸、第2和第3个苷酸之间。
ttcaagggaaaaagaaaaggg

SEQ ID NO: 40 - RNA, 21 nt, synthetic construct
  source 1..21: mol_type = other RNA; note; note (original language) = 5'端带有乙烯基磷酸二酯基。第2、6、12、14、16位为2'-氟代修饰；其余位置为2'-甲氧基修饰。硫代磷酸二酯基位于5'端第1和第2核苷酸、第2和第3核苷酸之间；3'端第1和第2核苷酸、第2和第3个苷酸之间。
tcaagggaaaaagaaaaggga

SEQ ID NO: 41 - RNA, 21 nt, synthetic construct
  source 1..21: mol_type = other RNA; note; note (original language) = 第2、4、6、10、12、14、16、18位为2'-氟代修饰；其余位置为2'-甲氧基修饰。硫代磷酸二酯基位于5'端第1和第2核苷酸、第2和第3核苷酸之间；3'端第1和第2核苷酸、第2和第3个苷酸之间。
ttgatgctgatgctgacagca

SEQ ID NO: 42 - RNA, 21 nt, synthetic construct
  source 1..21: mol_type = other RNA; note; note (original language) = 第2、4、6、10、12、14、16、18位为2'-氟代修饰；其余位置为2'-甲氧基修饰。硫代磷酸二酯基位于5'端第1和第2核苷酸、第2和第3核苷酸之间；3'端第1和第2核苷酸、第2和第3个苷酸之间。
ttacaggagagagttggtctg

SEQ ID NO: 43 - RNA, 21 nt, synthetic construct
  source 1..21: mol_type = other RNA; note; note (original language) = 第2、4、6、10、12、14、16、18位为2'-氟代修饰；其余位置为2'-甲氧基修饰。硫代磷酸二酯基位于5'端第1和第2核苷酸、第2和第3核苷酸之间；3'端第1和第2核苷酸、第2和第3个苷酸之间。
ttctgcacgctcctcctcttc

SEQ ID NO: 44 - RNA, 21 nt, synthetic construct
  source 1..21: mol_type = other RNA; note; note (original language) = 第2、4、6、10、12、14、16、18位为2'-氟代修饰；其余位置为2'-甲氧基修饰。硫代磷酸二酯基位于5'端第1和第2核苷酸、第2和第3核苷酸之间；3'端第1和第2核苷酸、第2和第3个苷酸之间。
tcaccattagctccgactgca

SEQ ID NO: 45 - RNA, 21 nt, synthetic construct
  source 1..21: mol_type = other RNA; note; note (original language) = 第2、4、6、10、12、14、16、18位为2'-氟代修饰；其余位置为2'-甲氧基修饰。硫代磷酸二酯基位于5'端第1和第2核苷酸、第2和第3核苷酸之间；3'端第1和第2核苷酸、第2和第3个苷酸之间。
ttcaagggaaaaagaaaaggg

SEQ ID NO: 46 - RNA, 21 nt, synthetic construct
  source 1..21: mol_type = other RNA; note; note (original language) = 第2、4、6、10、12、14、16位为2'-氟代修饰；其余位置为2'-甲氧基修饰。硫代磷酸二酯基位于5'端第1和第2核苷酸、第2和第3核苷酸之间；3'端第1和第2核苷酸、第2和第3个苷酸之间。
tcaagggaaaaagaaaaggga

SEQ ID NO: 47 - RNA, 21 nt, synthetic construct
  source 1..21: mol_type = other RNA; note; note (original language) = 第2、4、6、10、12、14、16、18位为2'-氟代修饰；其余位置为2'-甲氧基修饰。硫代磷酸二酯基位于5'端第1和第2核苷酸、第2和第3核苷酸之间；3'端第1和第2核苷酸、第2和第3个苷酸之间。
ttgatgctgatgctgacagca

SEQ ID NO: 48 - RNA, 21 nt, synthetic construct
  source 1..21: mol_type = other RNA; note; note (original language) = 第2、4、6、10、12、14、16、18位为2'-氟代修饰；其余位置为2'-甲氧基修饰。硫代磷酸二酯基位于5'端第1和第2核苷酸、第2和第3核苷酸之间；3'端第1和第2核苷酸、第2和第3个
ttacaggagagagttggtctg

SEQ ID NO: 49 - RNA, 21 nt, synthetic construct
  source 1..21: mol_type = other RNA; note; note (original language) = 第2、4、6、10、12、14、16、18位为2'-氟代修饰；其余位置为2'-甲氧基修饰。硫代磷酸二酯基位于5'端第1和第2核苷酸、第2和第3核苷酸之间；3'端第1和第2核苷酸、第2和第3个苷酸之间。
ttctgcacgctcctcctcttc

SEQ ID NO: 50 - RNA, 21 nt, synthetic construct
  source 1..21: mol_type = other RNA; note; note (original language) = 第2、4、6、10、12、14、16、18位为2'-氟代修饰；其余位置为2'-甲氧基修饰。硫代磷酸二酯基位于5'端第1和第2核苷酸、第2和第3核苷酸之间；3'端第1和第2核苷酸、第2和第3个苷酸之间。
tcaccattagctccgactgca

SEQ ID NO: 51 - RNA, 21 nt, synthetic construct
  source 1..21: mol_type = other RNA; note; note (original language) = 第2、4、6、10、12、14、16、18位为2'-氟代修饰；其余位置为2'-甲氧基修饰。硫代磷酸二酯基位于5'端第1和第2核苷酸、第2和第3核苷酸之间；3'端第1和第2核苷酸、第2和第3个苷酸之间。
ttcaagggaaaaagaaaaggg

SEQ ID NO: 52 - RNA, 21 nt, synthetic construct
  source 1..21: mol_type = other RNA; note; note (original language) = 第2、4、6、10、12、14、16位为2'-氟代修饰；其余位置为2'-甲氧基修饰。硫代磷酸二酯基位于5'端第1和第2核苷酸、第2和第3核苷酸之间；3'端第1和第2核苷酸、第2和第3个苷酸之间。
tcaagggaaaaagaaaaggga

SEQ ID NO: 53 - RNA, 19 nt, Homo sapiens
  source 1..19: mol_type = mRNA
gggcagtagtaggtgctca

SEQ ID NO: 54 - RNA, 19 nt, Homo sapiens
  source 1..19: mol_type = mRNA
ggcagtagtaggtgctcaa

SEQ ID NO: 55 - RNA, 19 nt, Homo sapiens
  source 1..19: mol_type = mRNA
gcagtagtaggtgctcaaa

SEQ ID NO: 56 - RNA, 19 nt, Homo sapiens
  source 1..19: mol_type = mRNA
cagtagtaggtgctcaaaa

SEQ ID NO: 57 - RNA, 19 nt, Homo sapiens
  source 1..19: mol_type = mRNA
ctgtcgggatccaggatga

SEQ ID NO: 58 - RNA, 19 nt, Homo sapiens
  source 1..19: mol_type = mRNA
cggtgccaggcaatgaaca

SEQ ID NO: 59 - RNA, 19 nt, Homo sapiens
  source 1..19: mol_type = mRNA
gccaggcaatgaacaggaa

SEQ ID NO: 60 - RNA, 19 nt, Homo sapiens
  source 1..19: mol_type = mRNA
ggaatggaaaggagaccaa

SEQ ID NO: 61 - RNA, 19 nt, Homo sapiens
  source 1..19: mol_type = mRNA
ggaaaggagaccaagtcca

SEQ ID NO: 62 - RNA, 19 nt, Homo sapiens
  source 1..19: mol_type = mRNA
gaaaggagaccaagtccaa

SEQ ID NO: 63 - RNA, 19 nt, Homo sapiens
  source 1..19: mol_type = mRNA
aggagaccaagtccaacta

SEQ ID NO: 64 - RNA, 19 nt, Homo sapiens
  source 1..19: mol_type = mRNA
gaccaagtccaactaccga

SEQ ID NO: 65 - RNA, 19 nt, Homo sapiens
  source 1..19: mol_type = mRNA
cacggctggtgttcccaat

SEQ ID NO: 66 - RNA, 19 nt, Homo sapiens
  source 1..19: mol_type = mRNA
acatgtgtgtcagagggaa

SEQ ID NO: 67 - RNA, 19 nt, Homo sapiens
  source 1..19: mol_type = mRNA
gtgtgtcagagggaagcta

SEQ ID NO: 68 - RNA, 19 nt, Homo sapiens
  source 1..19: mol_type = mRNA
cccctggtgcctaatgaga

SEQ ID NO: 69 - RNA, 19 nt, Homo sapiens
  source 1..19: mol_type = mRNA
ccctggtgcctaatgagaa

SEQ ID NO: 70 - RNA, 19 nt, Homo sapiens
  source 1..19: mol_type = mRNA
gggagtatctgtgaaggaa

SEQ ID NO: 71 - RNA, 19 nt, Homo sapiens
  source 1..19: mol_type = mRNA
caggagacaccctgagaca

SEQ ID NO: 72 - RNA, 19 nt, Homo sapiens
  source 1..19: mol_type = mRNA
acactgcagtcggagctaa

SEQ ID NO: 73 - RNA, 19 nt, Homo sapiens
  source 1..19: mol_type = mRNA
cactgcagtcggagctaat

SEQ ID NO: 74 - RNA, 19 nt, Homo sapiens
  source 1..19: mol_type = mRNA
gccagaaggtggagcagta

SEQ ID NO: 75 - RNA, 19 nt, Homo sapiens
  source 1..19: mol_type = mRNA
gcagtagctcctggtggaa

SEQ ID NO: 76 - RNA, 19 nt, Homo sapiens
  source 1..19: mol_type = mRNA
gctcctggtggaaccgtaa

SEQ ID NO: 77 - RNA, 19 nt, Homo sapiens
  source 1..19: mol_type = mRNA
ggtggaaccgtaaccctga

SEQ ID NO: 78 - RNA, 19 nt, Homo sapiens
  source 1..19: mol_type = mRNA
ccgtaaccctgacctgtga

SEQ ID NO: 79 - RNA, 19 nt, Homo sapiens
  source 1..19: mol_type = mRNA
cgtaaccctgacctgtgaa

SEQ ID NO: 80 - RNA, 19 nt, Homo sapiens
  source 1..19: mol_type = mRNA
ctgtgctgatcctccctga

SEQ ID NO: 81 - RNA, 19 nt, Homo sapiens
  source 1..19: mol_type = mRNA
gctgatcctccctgagata

SEQ ID NO: 82 - RNA, 19 nt, Homo sapiens
  source 1..19: mol_type = mRNA
caggaaagccgtgctgtca

SEQ ID NO: 83 - RNA, 19 nt, Homo sapiens
  source 1..19: mol_type = mRNA
cgtgctgtcagcatcagca

SEQ ID NO: 84 - RNA, 19 nt, Homo sapiens
  source 1..19: mol_type = mRNA
gcatcatcgaaccaggcga

SEQ ID NO: 85 - RNA, 19 nt, Homo sapiens
  source 1..19: mol_type = mRNA
ggggtcatcttgtggcaaa

SEQ ID NO: 86 - RNA, 19 nt, Homo sapiens
  source 1..19: mol_type = mRNA
ctttttcccttgaactgtt

SEQ ID NO: 87 - RNA, 19 nt, Homo sapiens
  source 1..19: mol_type = mRNA
ccaactctctcctgtataa

SEQ ID NO: 88 - RNA, 19 nt, Homo sapiens
  source 1..19: mol_type = mRNA
ggctgtcgggatccaggat

SEQ ID NO: 89 - RNA, 19 nt, Homo sapiens
  source 1..19: mol_type = mRNA
ggaagcccctggtgcctaa

SEQ ID NO: 90 - RNA, 19 nt, Homo sapiens
  source 1..19: mol_type = mRNA
gcctctggaggaggtccaa

SEQ ID NO: 91 - RNA, 19 nt, Homo sapiens
  source 1..19: mol_type = mRNA
gcccagccctctcctcaaa

SEQ ID NO: 92 - RNA, 19 nt, Homo sapiens
  source 1..19: mol_type = mRNA
ggaagaggaggagcgtgca

SEQ ID NO: 93 - RNA, 19 nt, Homo sapiens
  source 1..19: mol_type = mRNA
caaccagagccccccacaa

SEQ ID NO: 94 - RNA, 19 nt, Homo sapiens
  source 1..19: mol_type = mRNA
ccagagccccccacaatga

SEQ ID NO: 95 - RNA, 19 nt, Homo sapiens
  source 1..19: mol_type = mRNA
ctgggacagtgtggctcgt

SEQ ID NO: 96 - RNA, 19 nt, Homo sapiens
  source 1..19: mol_type = mRNA
agtccaactaccgagtcca

SEQ ID NO: 97 - RNA, 19 nt, Homo sapiens
  source 1..19: mol_type = mRNA
gtccaactaccgagtccgt

SEQ ID NO: 98 - RNA, 19 nt, Homo sapiens
  source 1..19: mol_type = mRNA
catcacagcccggattgga

SEQ ID NO: 99 - RNA, 19 nt, Homo sapiens
  source 1..19: mol_type = mRNA
aaggtggggacatgtgtgt

SEQ ID NO: 100 - RNA, 19 nt, Homo sapiens
  source 1..19: mol_type = mRNA
aggtggggacatgtgtgta

SEQ ID NO: 101 - RNA, 19 nt, Homo sapiens
  source 1..19: mol_type = mRNA
ggtggggacatgtgtgtca

SEQ ID NO: 102 - RNA, 19 nt, Homo sapiens
  source 1..19: mol_type = mRNA
ggaagctaccctgcaggga

SEQ ID NO: 103 - RNA, 19 nt, Homo sapiens
  source 1..19: mol_type = mRNA
gaagctaccctgcagggaa

SEQ ID NO: 104 - RNA, 19 nt, Homo sapiens
  source 1..19: mol_type = mRNA
aagctaccctgcagggact

SEQ ID NO: 105 - RNA, 19 nt, Homo sapiens
  source 1..19: mol_type = mRNA
accaggagacaccctgaga

SEQ ID NO: 106 - RNA, 19 nt, Homo sapiens
  source 1..19: mol_type = mRNA
ccaggagacaccctgagaa

SEQ ID NO: 107 - RNA, 21 nt, Homo sapiens
  source 1..21: mol_type = mRNA
tgagcacctactactgccccc

SEQ ID NO: 108 - RNA, 21 nt, Homo sapiens
  source 1..21: mol_type = mRNA
ttgagcacctactactgcccc

SEQ ID NO: 109 - RNA, 21 nt, Homo sapiens
  source 1..21: mol_type = mRNA
tttgagcacctactactgccc

SEQ ID NO: 110 - RNA, 21 nt, Homo sapiens
  source 1..21: mol_type = mRNA
ttttgagcacctactactgcc

SEQ ID NO: 111 - RNA, 21 nt, Homo sapiens
  source 1..21: mol_type = mRNA
tcatcctggatcccgacagcc

SEQ ID NO: 112 - RNA, 21 nt, Homo sapiens
  source 1..21: mol_type = mRNA
tgttcattgcctggcaccgga

SEQ ID NO: 113 - RNA, 21 nt, Homo sapiens
  source 1..21: mol_type = mRNA
ttcctgttcattgcctggcac

SEQ ID NO: 114 - RNA, 21 nt, Homo sapiens
  source 1..21: mol_type = mRNA
ttggtctcctttccattcctg

SEQ ID NO: 115 - RNA, 21 nt, Homo sapiens
  source 1..21: mol_type = mRNA
tggacttggtctcctttccat

SEQ ID NO: 116 - RNA, 21 nt, Homo sapiens
  source 1..21: mol_type = mRNA
ttggacttggtctcctttcca

SEQ ID NO: 117 - RNA, 21 nt, Homo sapiens
  source 1..21: mol_type = mRNA
tagttggacttggtctccttt

SEQ ID NO: 118 - RNA, 21 nt, Homo sapiens
  source 1..21: mol_type = mRNA
tcggtagttggacttggtctc

SEQ ID NO: 119 - RNA, 21 nt, Homo sapiens
  source 1..21: mol_type = mRNA
attgggaacaccagccgtgag

SEQ ID NO: 120 - RNA, 21 nt, Homo sapiens
  source 1..21: mol_type = mRNA
ttccctctgacacacatgtcc

SEQ ID NO: 121 - RNA, 21 nt, Homo sapiens
  source 1..21: mol_type = mRNA
tagcttccctctgacacacat

SEQ ID NO: 122 - RNA, 21 nt, Homo sapiens
  source 1..21: mol_type = mRNA
tctcattaggcaccaggggct

SEQ ID NO: 123 - RNA, 21 nt, Homo sapiens
  source 1..21: mol_type = mRNA
ttctcattaggcaccaggggc

SEQ ID NO: 124 - RNA, 21 nt, Homo sapiens
  source 1..21: mol_type = mRNA
ttccttcacagatactccctt

SEQ ID NO: 125 - RNA, 21 nt, Homo sapiens
  source 1..21: mol_type = mRNA
tgtctcagggtgtctcctggt

SEQ ID NO: 126 - RNA, 21 nt, Homo sapiens
  source 1..21: mol_type = mRNA
ttagctccgactgcagtgtga

SEQ ID NO: 127 - RNA, 21 nt, Homo sapiens
  source 1..21: mol_type = mRNA
attagctccgactgcagtgtg

SEQ ID NO: 128 - RNA, 21 nt, Homo sapiens
  source 1..21: mol_type = mRNA
tactgctccaccttctggctc

SEQ ID NO: 129 - RNA, 21 nt, Homo sapiens
  source 1..21: mol_type = mRNA
ttccaccaggagctactgctc

SEQ ID NO: 130 - RNA, 21 nt, Homo sapiens
  source 1..21: mol_type = mRNA
ttacggttccaccaggagcta

SEQ ID NO: 131 - RNA, 21 nt, Homo sapiens
  source 1..21: mol_type = mRNA
tcagggttacggttccaccag

SEQ ID NO: 132 - RNA, 21 nt, Homo sapiens
  source 1..21: mol_type = mRNA
tcacaggtcagggttacggtt

SEQ ID NO: 133 - RNA, 21 nt, Homo sapiens
  source 1..21: mol_type = mRNA
ttcacaggtcagggttacggt

SEQ ID NO: 134 - RNA, 21 nt, Homo sapiens
  source 1..21: mol_type = mRNA
tcagggaggatcagcacaggg

SEQ ID NO: 135 - RNA, 21 nt, Homo sapiens
  source 1..21: mol_type = mRNA
tatctcagggaggatcagcac

SEQ ID NO: 136 - RNA, 21 nt, Homo sapiens
  source 1..21: mol_type = mRNA
tgacagcacggctttcctggg

SEQ ID NO: 137 - RNA, 21 nt, Homo sapiens
  source 1..21: mol_type = mRNA
tgctgatgctgacagcacggc

SEQ ID NO: 138 - RNA, 21 nt, Homo sapiens
  source 1..21: mol_type = mRNA
tcgcctggttcgatgatgctg

SEQ ID NO: 139 - RNA, 21 nt, Homo sapiens
  source 1..21: mol_type = mRNA
tttgccacaagatgaccccaa

SEQ ID NO: 140 - RNA, 21 nt, Homo sapiens
  source 1..21: mol_type = mRNA
aacagttcaagggaaaaagaa

SEQ ID NO: 141 - RNA, 21 nt, Homo sapiens
  source 1..21: mol_type = mRNA
ttatacaggagagagttggtc

SEQ ID NO: 142 - RNA, 21 nt, Homo sapiens
  source 1..21: mol_type = mRNA
atcctggatcccgacagccgg

SEQ ID NO: 143 - RNA, 21 nt, Homo sapiens
  source 1..21: mol_type = mRNA
ttaggcaccaggggcttccca

SEQ ID NO: 144 - RNA, 21 nt, Homo sapiens
  source 1..21: mol_type = mRNA
ttggacctcctccagaggcac

SEQ ID NO: 145 - RNA, 21 nt, Homo sapiens
  source 1..21: mol_type = mRNA
tttgaggagagggctgggcag

SEQ ID NO: 146 - RNA, 21 nt, Homo sapiens
  source 1..21: mol_type = mRNA
tgcacgctcctcctcttcctc

SEQ ID NO: 147 - RNA, 21 nt, Homo sapiens
  source 1..21: mol_type = mRNA
ttgtggggggctctggttgta

SEQ ID NO: 148 - RNA, 21 nt, Homo sapiens
  source 1..21: mol_type = mRNA
tcattgtggggggctctggtt

SEQ ID NO: 149 - RNA, 21 nt, Homo sapiens
  source 1..21: mol_type = mRNA
acgagccacactgtcccaggg

SEQ ID NO: 150 - RNA, 21 nt, Homo sapiens
  source 1..21: mol_type = mRNA
tggactcggtagttggacttg

SEQ ID NO: 151 - RNA, 21 nt, Homo sapiens
  source 1..21: mol_type = mRNA
acggactcggtagttggactt

SEQ ID NO: 152 - RNA, 21 nt, Homo sapiens
  source 1..21: mol_type = mRNA
tccaatccgggctgtgatgtt

SEQ ID NO: 153 - RNA, 21 nt, Homo sapiens
  source 1..21: mol_type = mRNA
acacacatgtccccaccttat

SEQ ID NO: 154 - RNA, 21 nt, Homo sapiens
  source 1..21: mol_type = mRNA
tacacacatgtccccacctta

SEQ ID NO: 155 - RNA, 21 nt, Homo sapiens
  source 1..21: mol_type = mRNA
tgacacacatgtccccacctt

SEQ ID NO: 156 - RNA, 21 nt, Homo sapiens
  source 1..21: mol_type = mRNA
tccctgcagggtagcttccct

SEQ ID NO: 157 - RNA, 21 nt, Homo sapiens
  source 1..21: mol_type = mRNA
ttccctgcagggtagcttccc

SEQ ID NO: 158 - RNA, 21 nt, Homo sapiens
  source 1..21: mol_type = mRNA
agtccctgcagggtagcttcc

SEQ ID NO: 159 - RNA, 21 nt, Homo sapiens
  source 1..21: mol_type = mRNA
tctcagggtgtctcctggtct

SEQ ID NO: 160 - RNA, 21 nt, Homo sapiens
  source 1..21: mol_type = mRNA
ttctcagggtgtctcctggtc

SEQ ID NO: 161 - RNA, 19 nt, synthetic construct
  source 1..19: mol_type = other RNA; note; note (original language) = 第7-9位为2'-氟代修饰；其余位置为2'-甲氧基修饰。硫代磷酸二酯基位于5'端第1和第2核苷酸、第2和第3核苷酸之间。
gggcagtagtaggtgctca

SEQ ID NO: 162 - RNA, 19 nt, synthetic construct
  source 1..19: mol_type = other RNA; note; note (original language) = 第7-9位为2'-氟代修饰；其余位置为2'-甲氧基修饰。硫代磷酸二酯基位于5'端第1和第2核苷酸、第2和第3核苷酸之间。
ggcagtagtaggtgctcaa

SEQ ID NO: 163 - RNA, 19 nt, synthetic construct
  source 1..19: mol_type = other RNA; note; note (original language) = 第7-9位为2'-氟代修饰；其余位置为2'-甲氧基修饰。硫代磷酸二酯基位于5'端第1和第2核苷酸、第2和第3核苷酸之间。
gcagtagtaggtgctcaaa

SEQ ID NO: 164 - RNA, 19 nt, synthetic construct
  source 1..19: mol_type = other RNA; note; note (original language) = 第7-9位为2'-氟代修饰；其余位置为2'-甲氧基修饰。硫代磷酸二酯基位于5'端第1和第2核苷酸、第2和第3核苷酸之间。
cagtagtaggtgctcaaaa

SEQ ID NO: 165 - RNA, 19 nt, synthetic construct
  source 1..19: mol_type = other RNA; note; note (original language) = 第7-9位为2'-氟代修饰；其余位置为2'-甲氧基修饰。硫代磷酸二酯基位于5'端第1和第2核苷酸、第2和第3核苷酸之间。
ctgtcgggatccaggatga

SEQ ID NO: 166 - RNA, 19 nt, synthetic construct
  source 1..19: mol_type = other RNA; note; note (original language) = 第7-9位为2'-氟代修饰；其余位置为2'-甲氧基修饰。硫代磷酸二酯基位于5'端第1和第2核苷酸、第2和第3核苷酸之间。
cggtgccaggcaatgaaca

SEQ ID NO: 167 - RNA, 19 nt, synthetic construct
  source 1..19: mol_type = other RNA; note; note (original language) = 第7-9位为2'-氟代修饰；其余位置为2'-甲氧基修饰。硫代磷酸二酯基位于5'端第1和第2核苷酸、第2和第3核苷酸之间。
gccaggcaatgaacaggaa

SEQ ID NO: 168 - RNA, 19 nt, synthetic construct
  source 1..19: mol_type = other RNA; note; note (original language) = 第7-9位为2'-氟代修饰；其余位置为2'-甲氧基修饰。硫代磷酸二酯基位于5'端第1和第2核苷酸、第2和第3核苷酸之间。
ggaatggaaaggagaccaa

SEQ ID NO: 169 - RNA, 19 nt, synthetic construct
  source 1..19: mol_type = other RNA; note; note (original language) = 第7-9位为2'-氟代修饰；其余位置为2'-甲氧基修饰。硫代磷酸二酯基位于5'端第1和第2核苷酸、第2和第3核苷酸之间。
ggaaaggagaccaagtcca

SEQ ID NO: 170 - RNA, 19 nt, synthetic construct
  source 1..19: mol_type = other RNA; note; note (original language) = 第7-9位为2'-氟代修饰；其余位置为2'-甲氧基修饰。硫代磷酸二酯基位于5'端第1和第2核苷酸、第2和第3核苷酸之间。
gaaaggagaccaagtccaa

SEQ ID NO: 171 - RNA, 19 nt, synthetic construct
  source 1..19: mol_type = other RNA; note; note (original language) = 第7-9位为2'-氟代修饰；其余位置为2'-甲氧基修饰。硫代磷酸二酯基位于5'端第1和第2核苷酸、第2和第3核苷酸之间。
aggagaccaagtccaacta

SEQ ID NO: 172 - RNA, 19 nt, synthetic construct
  source 1..19: mol_type = other RNA; note; note (original language) = 第7-9位为2'-氟代修饰；其余位置为2'-甲氧基修饰。硫代磷酸二酯基位于5'端第1和第2核苷酸、第2和第3核苷酸之间。
gaccaagtccaactaccga

SEQ ID NO: 173 - RNA, 19 nt, synthetic construct
  source 1..19: mol_type = other RNA; note; note (original language) = 第7-9位为2'-氟代修饰；其余位置为2'-甲氧基修饰。硫代磷酸二酯基位于5'端第1和第2核苷酸、第2和第3核苷酸之间。
cacggctggtgttcccaaa

SEQ ID NO: 174 - RNA, 19 nt, synthetic construct
  source 1..19: mol_type = other RNA; note; note (original language) = 第7-9位为2'-氟代修饰；其余位置为2'-甲氧基修饰。硫代磷酸二酯基位于5'端第1和第2核苷酸、第2和第3核苷酸之间。
acatgtgtgtcagagggaa

SEQ ID NO: 175 - RNA, 19 nt, synthetic construct
  source 1..19: mol_type = other RNA; note; note (original language) = 第7-9位为2'-氟代修饰；其余位置为2'-甲氧基修饰。硫代磷酸二酯基位于5'端第1和第2核苷酸、第2和第3核苷酸之间。
gtgtgtcagagggaagcta

SEQ ID NO: 176 - RNA, 19 nt, synthetic construct
  source 1..19: mol_type = other RNA; note; note (original language) = 第7-9位为2'-氟代修饰；其余位置为2'-甲氧基修饰。硫代磷酸二酯基位于5'端第1和第2核苷酸、第2和第3核苷酸之间。
cccctggtgcctaatgaga

SEQ ID NO: 177 - RNA, 19 nt, synthetic construct
  source 1..19: mol_type = other RNA; note; note (original language) = 第7-9位为2'-氟代修饰；其余位置为2'-甲氧基修饰。硫代磷酸二酯基位于5'端第1和第2核苷酸、第2和第3核苷酸之间。
ccctggtgcctaatgagaa

SEQ ID NO: 178 - RNA, 19 nt, synthetic construct
  source 1..19: mol_type = other RNA; note; note (original language) = 第7-9位为2'-氟代修饰；其余位置为2'-甲氧基修饰。硫代磷酸二酯基位于5'端第1和第2核苷酸、第2和第3核苷酸之间。
gggagtatctgtgaaggaa

SEQ ID NO: 179 - RNA, 19 nt, synthetic construct
  source 1..19: mol_type = other RNA; note; note (original language) = 第7-9位为2'-氟代修饰；其余位置为2'-甲氧基修饰。硫代磷酸二酯基位于5'端第1和第2核苷酸、第2和第3核苷酸之间。
caggagacaccctgagaca

SEQ ID NO: 180 - RNA, 19 nt, synthetic construct
  source 1..19: mol_type = other RNA; note; note (original language) = 第7-9位为2'-氟代修饰；其余位置为2'-甲氧基修饰。硫代磷酸二酯基位于5'端第1和第2核苷酸、第2和第3核苷酸之间。
acactgcagtcggagctaa

SEQ ID NO: 181 - RNA, 19 nt, synthetic construct
  source 1..19: mol_type = other RNA; note; note (original language) = 第7-9位为2'-氟代修饰；其余位置为2'-甲氧基修饰。硫代磷酸二酯基位于5'端第1和第2核苷酸、第2和第3核苷酸之间。
cactgcagtcggagctaaa

SEQ ID NO: 182 - RNA, 19 nt, synthetic construct
  source 1..19: mol_type = other RNA; note; note (original language) = 第7-9位为2'-氟代修饰；其余位置为2'-甲氧基修饰。硫代磷酸二酯基位于5'端第1和第2核苷酸、第2和第3核苷酸之间。
gccagaaggtggagcagta

SEQ ID NO: 183 - RNA, 19 nt, synthetic construct
  source 1..19: mol_type = other RNA; note; note (original language) = 第7-9位为2'-氟代修饰；其余位置为2'-甲氧基修饰。硫代磷酸二酯基位于5'端第1和第2核苷酸、第2和第3核苷酸之间。
gcagtagctcctggtggaa

SEQ ID NO: 184 - RNA, 19 nt, synthetic construct
  source 1..19: mol_type = other RNA; note; note (original language) = 第7-9位为2'-氟代修饰；其余位置为2'-甲氧基修饰。硫代磷酸二酯基位于5'端第1和第2核苷酸、第2和第3核苷酸之间。
gctcctggtggaaccgtaa

SEQ ID NO: 185 - RNA, 19 nt, synthetic construct
  source 1..19: mol_type = other RNA; note; note (original language) = 第7-9位为2'-氟代修饰；其余位置为2'-甲氧基修饰。硫代磷酸二酯基位于5'端第1和第2核苷酸、第2和第3核苷酸之间。
ggtggaaccgtaaccctga

SEQ ID NO: 186 - RNA, 19 nt, synthetic construct
  source 1..19: mol_type = other RNA; note; note (original language) = 第7-9位为2'-氟代修饰；其余位置为2'-甲氧基修饰。硫代磷酸二酯基位于5'端第1和第2核苷酸、第2和第3核苷酸之间。
ccgtaaccctgacctgtga

SEQ ID NO: 187 - RNA, 19 nt, synthetic construct
  source 1..19: mol_type = other RNA; note; note (original language) = 第7-9位为2'-氟代修饰；其余位置为2'-甲氧基修饰。硫代磷酸二酯基位于5'端第1和第2核苷酸、第2和第3核苷酸之间。
cgtaaccctgacctgtgaa

SEQ ID NO: 188 - RNA, 19 nt, synthetic construct
  source 1..19: mol_type = other RNA; note; note (original language) = 第7-9位为2'-氟代修饰；其余位置为2'-甲氧基修饰。硫代磷酸二酯基位于5'端第1和第2核苷酸、第2和第3核苷酸之间。
ctgtgctgatcctccctga

SEQ ID NO: 189 - RNA, 19 nt, synthetic construct
  source 1..19: mol_type = other RNA; note; note (original language) = 第7-9位为2'-氟代修饰；其余位置为2'-甲氧基修饰。硫代磷酸二酯基位于5'端第1和第2核苷酸、第2和第3核苷酸之间。
gctgatcctccctgagata

SEQ ID NO: 190 - RNA, 19 nt, synthetic construct
  source 1..19: mol_type = other RNA; note; note (original language) = 第7-9位为2'-氟代修饰；其余位置为2'-甲氧基修饰。硫代磷酸二酯基位于5'端第1和第2核苷酸、第2和第3核苷酸之间。
caggaaagccgtgctgtca

SEQ ID NO: 191 - RNA, 19 nt, synthetic construct
  source 1..19: mol_type = other RNA; note; note (original language) = 第7-9位为2'-氟代修饰；其余位置为2'-甲氧基修饰。硫代磷酸二酯基位于5'端第1和第2核苷酸、第2和第3核苷酸之间。
cgtgctgtcagcatcagca

SEQ ID NO: 192 - RNA, 19 nt, synthetic construct
  source 1..19: mol_type = other RNA; note; note (original language) = 第7-9位为2'-氟代修饰；其余位置为2'-甲氧基修饰。硫代磷酸二酯基位于5'端第1和第2核苷酸、第2和第3核苷酸之间。
gcatcatcgaaccaggcga

SEQ ID NO: 193 - RNA, 19 nt, synthetic construct
  source 1..19: mol_type = other RNA; note; note (original language) = 第7-9位为2'-氟代修饰；其余位置为2'-甲氧基修饰。硫代磷酸二酯基位于5'端第1和第2核苷酸、第2和第3核苷酸之间。
ggggtcatcttgtggcaaa

SEQ ID NO: 194 - RNA, 19 nt, synthetic construct
  source 1..19: mol_type = other RNA; note; note (original language) = 第7-9位为2'-氟代修饰；其余位置为2'-甲氧基修饰。硫代磷酸二酯基位于5'端第1和第2核苷酸、第2和第3核苷酸之间。
ctttttcccttgaactgta

SEQ ID NO: 195 - RNA, 19 nt, synthetic construct
  source 1..19: mol_type = other RNA; note; note (original language) = 第7-9位为2'-氟代修饰；其余位置为2'-甲氧基修饰。硫代磷酸二酯基位于5'端第1和第2核苷酸、第2和第3核苷酸之间。
ccaactctctcctgtataa

SEQ ID NO: 196 - RNA, 19 nt, synthetic construct
  source 1..19: mol_type = other RNA; note; note (original language) = 第7-9位为2'-氟代修饰；其余位置为2'-甲氧基修饰。硫代磷酸二酯基位于5'端第1和第2核苷酸、第2和第3核苷酸之间。
ggctgtcgggatccaggaa

SEQ ID NO: 197 - RNA, 19 nt, synthetic construct
  source 1..19: mol_type = other RNA; note; note (original language) = 第7-9位为2'-氟代修饰；其余位置为2'-甲氧基修饰。硫代磷酸二酯基位于5'端第1和第2核苷酸、第2和第3核苷酸之间。
ggaagcccctggtgcctaa

SEQ ID NO: 198 - RNA, 19 nt, synthetic construct
  source 1..19: mol_type = other RNA; note; note (original language) = 第7-9位为2'-氟代修饰；其余位置为2'-甲氧基修饰。硫代磷酸二酯基位于5'端第1和第2核苷酸、第2和第3核苷酸之间。
gcctctggaggaggtccaa

SEQ ID NO: 199 - RNA, 19 nt, synthetic construct
  source 1..19: mol_type = other RNA; note; note (original language) = 第7-9位为2'-氟代修饰；其余位置为2'-甲氧基修饰。硫代磷酸二酯基位于5'端第1和第2核苷酸、第2和第3核苷酸之间。
gcccagccctctcctcaaa

SEQ ID NO: 200 - RNA, 19 nt, synthetic construct
  source 1..19: mol_type = other RNA; note; note (original language) = 第7-9位为2'-氟代修饰；其余位置为2'-甲氧基修饰。硫代磷酸二酯基位于5'端第1和第2核苷酸、第2和第3核苷酸之间。
ggaagaggaggagcgtgca

SEQ ID NO: 201 - RNA, 19 nt, synthetic construct
  source 1..19: mol_type = other RNA; note; note (original language) = 第7-9位为2'-氟代修饰；其余位置为2'-甲氧基修饰。硫代磷酸二酯基位于5'端第1和第2核苷酸、第2和第3核苷酸之间。
caaccagagccccccacaa

SEQ ID NO: 202 - RNA, 19 nt, synthetic construct
  source 1..19: mol_type = other RNA; note; note (original language) = 第7-9位为2'-氟代修饰；其余位置为2'-甲氧基修饰。硫代磷酸二酯基位于5'端第1和第2核苷酸、第2和第3核苷酸之间。
ccagagccccccacaatga

SEQ ID NO: 203 - RNA, 19 nt, synthetic construct
  source 1..19: mol_type = other RNA; note; note (original language) = 第7-9位为2'-氟代修饰；其余位置为2'-甲氧基修饰。硫代磷酸二酯基位于5'端第1和第2核苷酸、第2和第3核苷酸之间。
ctgggacagtgtggctcga

SEQ ID NO: 204 - RNA, 19 nt, synthetic construct
  source 1..19: mol_type = other RNA; note; note (original language) = 第7-9位为2'-氟代修饰；其余位置为2'-甲氧基修饰。硫代磷酸二酯基位于5'端第1和第2核苷酸、第2和第3核苷酸之间。
agtccaactaccgagtcca

SEQ ID NO: 205 - RNA, 19 nt, synthetic construct
  source 1..19: mol_type = other RNA; note; note (original language) = 第7-9位为2'-氟代修饰；其余位置为2'-甲氧基修饰。硫代磷酸二酯基位于5'端第1和第2核苷酸、第2和第3核苷酸之间。
gtccaactaccgagtccga

SEQ ID NO: 206 - RNA, 19 nt, synthetic construct
  source 1..19: mol_type = other RNA; note; note (original language) = 第7-9位为2'-氟代修饰；其余位置为2'-甲氧基修饰。硫代磷酸二酯基位于5'端第1和第2核苷酸、第2和第3核苷酸之间。
catcacagcccggattgga

SEQ ID NO: 207 - RNA, 19 nt, synthetic construct
  source 1..19: mol_type = other RNA; note; note (original language) = 第7-9位为2'-氟代修饰；其余位置为2'-甲氧基修饰。硫代磷酸二酯基位于5'端第1和第2核苷酸、第2和第3核苷酸之间。
aaggtggggacatgtgtga

SEQ ID NO: 208 - RNA, 19 nt, synthetic construct
  source 1..19: mol_type = other RNA; note; note (original language) = 第7-9位为2'-氟代修饰；其余位置为2'-甲氧基修饰。硫代磷酸二酯基位于5'端第1和第2核苷酸、第2和第3核苷酸之间。
aggtggggacatgtgtgta

SEQ ID NO: 209 - RNA, 19 nt, synthetic construct
  source 1..19: mol_type = other RNA; note; note (original language) = 第7-9位为2'-氟代修饰；其余位置为2'-甲氧基修饰。硫代磷酸二酯基位于5'端第1和第2核苷酸、第2和第3核苷酸之间。
ggtggggacatgtgtgtca

SEQ ID NO: 210 - RNA, 19 nt, synthetic construct
  source 1..19: mol_type = other RNA; note; note (original language) = 第7-9位为2'-氟代修饰；其余位置为2'-甲氧基修饰。硫代磷酸二酯基位于5'端第1和第2核苷酸、第2和第3核苷酸之间。
ggaagctaccctgcaggga

SEQ ID NO: 211 - RNA, 19 nt, synthetic construct
  source 1..19: mol_type = other RNA; note; note (original language) = 第7-9位为2'-氟代修饰；其余位置为2'-甲氧基修饰。硫代磷酸二酯基位于5'端第1和第2核苷酸、第2和第3核苷酸之间。
gaagctaccctgcagggaa

SEQ ID NO: 212 - RNA, 19 nt, synthetic construct
  source 1..19: mol_type = other RNA; note; note (original language) = 第7-9位为2'-氟代修饰；其余位置为2'-甲氧基修饰。硫代磷酸二酯基位于5'端第1和第2核苷酸、第2和第3核苷酸之间。
aagctaccctgcagggaca

SEQ ID NO: 213 - RNA, 19 nt, synthetic construct
  source 1..19: mol_type = other RNA; note; note (original language) = 第7-9位为2'-氟代修饰；其余位置为2'-甲氧基修饰。硫代磷酸二酯基位于5'端第1和第2核苷酸、第2和第3核苷酸之间。
accaggagacaccctgaga

SEQ ID NO: 214 - RNA, 19 nt, synthetic construct
  source 1..19: mol_type = other RNA; note; note (original language) = 第7-9位为2'-氟代修饰；其余位置为2'-甲氧基修饰。硫代磷酸二酯基位于5'端第1和第2核苷酸、第2和第3核苷酸之间。
ccaggagacaccctgagaa

SEQ ID NO: 215 - RNA, 21 nt, synthetic construct
  source 1..21: mol_type = other RNA; note; note (original language) = 5'端带有乙烯基磷酸二酯基。第2、6、12、14、16位为2'-氟代修饰；其余位置为2'-甲氧基修饰。硫代磷酸二酯基位于5'端第1和第2核苷酸、第2和第3核苷酸之间；3'端第1和第2核苷酸、第2和第3个苷酸之间。
tgagcacctactactgccccc

SEQ ID NO: 216 - RNA, 21 nt, synthetic construct
  source 1..21: mol_type = other RNA; note; note (original language) = 5'端带有乙烯基磷酸二酯基。第2、6、12、14、16位为2'-氟代修饰；其余位置为2'-甲氧基修饰。硫代磷酸二酯基位于5'端第1和第2核苷酸、第2和第3核苷酸之间；3'端第1和第2核苷酸、第2和第3个苷酸之间。
ttgagcacctactactgcccc

SEQ ID NO: 217 - RNA, 21 nt, synthetic construct
  source 1..21: mol_type = other RNA; note; note (original language) = 5'端带有乙烯基磷酸二酯基。第2、6、12、14、16位为2'-氟代修饰；其余位置为2'-甲氧基修饰。硫代磷酸二酯基位于5'端第1和第2核苷酸、第2和第3核苷酸之间；3'端第1和第2核苷酸、第2和第3个苷酸之间。
tttgagcacctactactgccc

SEQ ID NO: 218 - RNA, 21 nt, synthetic construct
  source 1..21: mol_type = other RNA; note; note (original language) = 5'端带有乙烯基磷酸二酯基。第2、6、12、14、16位为2'-氟代修饰；其余位置为2'-甲氧基修饰。硫代磷酸二酯基位于5'端第1和第2核苷酸、第2和第3核苷酸之间；3'端第1和第2核苷酸、第2和第3个苷酸之间。
ttttgagcacctactactgcc

SEQ ID NO: 219 - RNA, 21 nt, synthetic construct
  source 1..21: mol_type = other RNA; note; note (original language) = 5'端带有乙烯基磷酸二酯基。第2、6、12、14、16位为2'-氟代修饰；其余位置为2'-甲氧基修饰。硫代磷酸二酯基位于5'端第1和第2核苷酸、第2和第3核苷酸之间；3'端第1和第2核苷酸、第2和第3个苷酸之间。
tcatcctggatcccgacagcc

SEQ ID NO: 220 - RNA, 21 nt, synthetic construct
  source 1..21: mol_type = other RNA; note; note (original language) = 5'端带有乙烯基磷酸二酯基。第2、6、12、14、16位为2'-氟代修饰；其余位置为2'-甲氧基修饰。硫代磷酸二酯基位于5'端第1和第2核苷酸、第2和第3核苷酸之间；3'端第1和第2核苷酸、第2和第3个苷酸之间。
tgttcattgcctggcaccgga

SEQ ID NO: 221 - RNA, 21 nt, synthetic construct
  source 1..21: mol_type = other RNA; note; note (original language) = 5'端带有乙烯基磷酸二酯基。第2、6、12、14、16位为2'-氟代修饰；其余位置为2'-甲氧基修饰。硫代磷酸二酯基位于5'端第1和第2核苷酸、第2和第3核苷酸之间；3'端第1和第2核苷酸、第2和第3个苷酸之间。
ttcctgttcattgcctggcac

SEQ ID NO: 222 - RNA, 21 nt, synthetic construct
  source 1..21: mol_type = other RNA; note; note (original language) = 5'端带有乙烯基磷酸二酯基。第2、6、12、14、16位为2'-氟代修饰；其余位置为2'-甲氧基修饰。硫代磷酸二酯基位于5'端第1和第2核苷酸、第2和第3核苷酸之间；3'端第1和第2核苷酸、第2和第3个苷酸之间。
ttggtctcctttccattcctg

SEQ ID NO: 223 - RNA, 21 nt, synthetic construct
  source 1..21: mol_type = other RNA; note; note (original language) = 5'端带有乙烯基磷酸二酯基。第2、6、12、14、16位为2'-氟代修饰；其余位置为2'-甲氧基修饰。硫代磷酸二酯基位于5'端第1和第2核苷酸、第2和第3核苷酸之间；3'端第1和第2核苷酸、第2和第3个苷酸之间。
tggacttggtctcctttccat

SEQ ID NO: 224 - RNA, 21 nt, synthetic construct
  source 1..21: mol_type = other RNA; note; note (original language) = 5'端带有乙烯基磷酸二酯基。第2、6、12、14、16位为2'-氟代修饰；其余位置为2'-甲氧基修饰。硫代磷酸二酯基位于5'端第1和第2核苷酸、第2和第3核苷酸之间；3'端第1和第2核苷酸、第2和第3个苷酸之间。
ttggacttggtctcctttcca

SEQ ID NO: 225 - RNA, 21 nt, synthetic construct
  source 1..21: mol_type = other RNA; note; note (original language) = 5'端带有乙烯基磷酸二酯基。第2、6、12、14、16位为2'-氟代修饰；其余位置为2'-甲氧基修饰。硫代磷酸二酯基位于5'端第1和第2核苷酸、第2和第3核苷酸之间；3'端第1和第2核苷酸、第2和第3个苷酸之间。
tagttggacttggtctccttt

SEQ ID NO: 226 - RNA, 21 nt, synthetic construct
  source 1..21: mol_type = other RNA; note; note (original language) = 5'端带有乙烯基磷酸二酯基。第2、6、12、14、16位为2'-氟代修饰；其余位置为2'-甲氧基修饰。硫代磷酸二酯基位于5'端第1和第2核苷酸、第2和第3核苷酸之间；3'端第1和第2核苷酸、第2和第3个苷酸之间。
tcggtagttggacttggtctc

SEQ ID NO: 227 - RNA, 21 nt, synthetic construct
  source 1..21: mol_type = other RNA; note; note (original language) = 5'端带有乙烯基磷酸二酯基。第2、6、12、14、16位为2'-氟代修饰；其余位置为2'-甲氧基修饰。硫代磷酸二酯基位于5'端第1和第2核苷酸、第2和第3核苷酸之间；3'端第1和第2核苷酸、第2和第3个苷酸之间。
tttgggaacaccagccgtgag

SEQ ID NO: 228 - RNA, 21 nt, synthetic construct
  source 1..21: mol_type = other RNA; note; note (original language) = 5'端带有乙烯基磷酸二酯基。第2、6、12、14、16位为2'-氟代修饰；其余位置为2'-甲氧基修饰。硫代磷酸二酯基位于5'端第1和第2核苷酸、第2和第3核苷酸之间；3'端第1和第2核苷酸、第2和第3个苷酸之间。
ttccctctgacacacatgtcc

SEQ ID NO: 229 - RNA, 21 nt, synthetic construct
  source 1..21: mol_type = other RNA; note; note (original language) = 5'端带有乙烯基磷酸二酯基。第2、6、12、14、16位为2'-氟代修饰；其余位置为2'-甲氧基修饰。硫代磷酸二酯基位于5'端第1和第2核苷酸、第2和第3核苷酸之间；3'端第1和第2核苷酸、第2和第3个苷酸之间。
tagcttccctctgacacacat

SEQ ID NO: 230 - RNA, 21 nt, synthetic construct
  source 1..21: mol_type = other RNA; note; note (original language) = 5'端带有乙烯基磷酸二酯基。第2、6、12、14、16位为2'-氟代修饰；其余位置为2'-甲氧基修饰。硫代磷酸二酯基位于5'端第1和第2核苷酸、第2和第3核苷酸之间；3'端第1和第2核苷酸、第2和第3个苷酸之间。
tctcattaggcaccaggggct

SEQ ID NO: 231 - RNA, 21 nt, synthetic construct
  source 1..21: mol_type = other RNA; note; note (original language) = 5'端带有乙烯基磷酸二酯基。第2、6、12、14、16位为2'-氟代修饰；其余位置为2'-甲氧基修饰。硫代磷酸二酯基位于5'端第1和第2核苷酸、第2和第3核苷酸之间；3'端第1和第2核苷酸、第2和第3个苷酸之间。
ttctcattaggcaccaggggc

SEQ ID NO: 232 - RNA, 21 nt, synthetic construct
  source 1..21: mol_type = other RNA; note; note (original language) = 5'端带有乙烯基磷酸二酯基。第2、6、12、14、16位为2'-氟代修饰；其余位置为2'-甲氧基修饰。硫代磷酸二酯基位于5'端第1和第2核苷酸、第2和第3核苷酸之间；3'端第1和第2核苷酸、第2和第3个苷酸之间。
ttccttcacagatactccctt

SEQ ID NO: 233 - RNA, 21 nt, synthetic construct
  source 1..21: mol_type = other RNA; note; note (original language) = 5'端带有乙烯基磷酸二酯基。第2、6、12、14、16位为2'-氟代修饰；其余位置为2'-甲氧基修饰。硫代磷酸二酯基位于5'端第1和第2核苷酸、第2和第3核苷酸之间；3'端第1和第2核苷酸、第2和第3个苷酸之间。
tgtctcagggtgtctcctggt

SEQ ID NO: 234 - RNA, 21 nt, synthetic construct
  source 1..21: mol_type = other RNA; note; note (original language) = 5'端带有乙烯基磷酸二酯基。第2、6、12、14、16位为2'-氟代修饰；其余位置为2'-甲氧基修饰。硫代磷酸二酯基位于5'端第1和第2核苷酸、第2和第3核苷酸之间；3'端第1和第2核苷酸、第2和第3个苷酸之间。
ttagctccgactgcagtgtga

SEQ ID NO: 235 - RNA, 21 nt, synthetic construct
  source 1..21: mol_type = other RNA; note; note (original language) = 5'端带有乙烯基磷酸二酯基。第2、6、12、14、16位为2'-氟代修饰；其余位置为2'-甲氧基修饰。硫代磷酸二酯基位于5'端第1和第2核苷酸、第2和第3核苷酸之间；3'端第1和第2核苷酸、第2和第3个苷酸之间。
tttagctccgactgcagtgtg

SEQ ID NO: 236 - RNA, 21 nt, synthetic construct
  source 1..21: mol_type = other RNA; note; note (original language) = 5'端带有乙烯基磷酸二酯基。第2、6、12、14、16位为2'-氟代修饰；其余位置为2'-甲氧基修饰。硫代磷酸二酯基位于5'端第1和第2核苷酸、第2和第3核苷酸之间；3'端第1和第2核苷酸、第2和第3个苷酸之间。
tactgctccaccttctggctc

SEQ ID NO: 237 - RNA, 21 nt, synthetic construct
  source 1..21: mol_type = other RNA; note; note (original language) = 5'端带有乙烯基磷酸二酯基。第2、6、12、14、16位为2'-氟代修饰；其余位置为2'-甲氧基修饰。硫代磷酸二酯基位于5'端第1和第2核苷酸、第2和第3核苷酸之间；3'端第1和第2核苷酸、第2和第3个苷酸之间。
ttccaccaggagctactgctc

SEQ ID NO: 238 - RNA, 21 nt, synthetic construct
  source 1..21: mol_type = other RNA; note; note (original language) = 5'端带有乙烯基磷酸二酯基。第2、6、12、14、16位为2'-氟代修饰；其余位置为2'-甲氧基修饰。硫代磷酸二酯基位于5'端第1和第2核苷酸、第2和第3核苷酸之间；3'端第1和第2核苷酸、第2和第3个苷酸之间。
ttacggttccaccaggagcta

SEQ ID NO: 239 - RNA, 21 nt, synthetic construct
  source 1..21: mol_type = other RNA; note; note (original language) = 5'端带有乙烯基磷酸二酯基。第2、6、12、14、16位为2'-氟代修饰；其余位置为2'-甲氧基修饰。硫代磷酸二酯基位于5'端第1和第2核苷酸、第2和第3核苷酸之间；3'端第1和第2核苷酸、第2和第3个苷酸之间。
tcagggttacggttccaccag

SEQ ID NO: 240 - RNA, 21 nt, synthetic construct
  source 1..21: mol_type = other RNA; note; note (original language) = 5'端带有乙烯基磷酸二酯基。第2、6、12、14、16位为2'-氟代修饰；其余位置为2'-甲氧基修饰。硫代磷酸二酯基位于5'端第1和第2核苷酸、第2和第3核苷酸之间；3'端第1和第2核苷酸、第2和第3个苷酸之间。
tcacaggtcagggttacggtt

SEQ ID NO: 241 - RNA, 21 nt, synthetic construct
  source 1..21: mol_type = other RNA; note; note (original language) = 5'端带有乙烯基磷酸二酯基。第2、6、12、14、16位为2'-氟代修饰；其余位置为2'-甲氧基修饰。硫代磷酸二酯基位于5'端第1和第2核苷酸、第2和第3核苷酸之间；3'端第1和第2核苷酸、第2和第3个苷酸之间。
ttcacaggtcagggttacggt

SEQ ID NO: 242 - RNA, 21 nt, synthetic construct
  source 1..21: mol_type = other RNA; note; note (original language) = 5'端带有乙烯基磷酸二酯基。第2、6、12、14、16位为2'-氟代修饰；其余位置为2'-甲氧基修饰。硫代磷酸二酯基位于5'端第1和第2核苷酸、第2和第3核苷酸之间；3'端第1和第2核苷酸、第2和第3个苷酸之间。
tcagggaggatcagcacaggg

SEQ ID NO: 243 - RNA, 21 nt, synthetic construct
  source 1..21: mol_type = other RNA; note; note (original language) = 5'端带有乙烯基磷酸二酯基。第2、6、12、14、16位为2'-氟代修饰；其余位置为2'-甲氧基修饰。硫代磷酸二酯基位于5'端第1和第2核苷酸、第2和第3核苷酸之间；3'端第1和第2核苷酸、第2和第3个苷酸之间。
tatctcagggaggatcagcac

SEQ ID NO: 244 - RNA, 21 nt, synthetic construct
  source 1..21: mol_type = other RNA; note; note (original language) = 5'端带有乙烯基磷酸二酯基。第2、6、12、14、16位为2'-氟代修饰；其余位置为2'-甲氧基修饰。硫代磷酸二酯基位于5'端第1和第2核苷酸、第2和第3核苷酸之间；3'端第1和第2核苷酸、第2和第3个苷酸之间。
tgacagcacggctttcctggg

SEQ ID NO: 245 - RNA, 21 nt, synthetic construct
  source 1..21: mol_type = other RNA; note; note (original language) = 5'端带有乙烯基磷酸二酯基。第2、6、12、14、16位为2'-氟代修饰；其余位置为2'-甲氧基修饰。硫代磷酸二酯基位于5'端第1和第2核苷酸、第2和第3核苷酸之间；3'端第1和第2核苷酸、第2和第3个苷酸之间。
tgctgatgctgacagcacggc

SEQ ID NO: 246 - RNA, 21 nt, synthetic construct
  source 1..21: mol_type = other RNA; note; note (original language) = 5'端带有乙烯基磷酸二酯基。第2、6、12、14、16位为2'-氟代修饰；其余位置为2'-甲氧基修饰。硫代磷酸二酯基位于5'端第1和第2核苷酸、第2和第3核苷酸之间；3'端第1和第2核苷酸、第2和第3个苷酸之间。
tcgcctggttcgatgatgctg

SEQ ID NO: 247 - RNA, 21 nt, synthetic construct
  source 1..21: mol_type = other RNA; note; note (original language) = 5'端带有乙烯基磷酸二酯基。第2、6、12、14、16位为2'-氟代修饰；其余位置为2'-甲氧基修饰。硫代磷酸二酯基位于5'端第1和第2核苷酸、第2和第3核苷酸之间；3'端第1和第2核苷酸、第2和第3个苷酸之间。
tttgccacaagatgaccccaa

SEQ ID NO: 248 - RNA, 21 nt, synthetic construct
  source 1..21: mol_type = other RNA; note; note (original language) = 5'端带有乙烯基磷酸二酯基。第2、6、12、14、16位为2'-氟代修饰；其余位置为2'-甲氧基修饰。硫代磷酸二酯基位于5'端第1和第2核苷酸、第2和第3核苷酸之间；3'端第1和第2核苷酸、第2和第3个苷酸之间。
tacagttcaagggaaaaagaa

SEQ ID NO: 249 - RNA, 21 nt, synthetic construct
  source 1..21: mol_type = other RNA; note; note (original language) = 5'端带有乙烯基磷酸二酯基。第2、6、12、14、16位为2'-氟代修饰；其余位置为2'-甲氧基修饰。硫代磷酸二酯基位于5'端第1和第2核苷酸、第2和第3核苷酸之间；3'端第1和第2核苷酸、第2和第3个苷酸之间。
ttatacaggagagagttggtc

SEQ ID NO: 250 - RNA, 21 nt, synthetic construct
  source 1..21: mol_type = other RNA; note; note (original language) = 5'端带有乙烯基磷酸二酯基。第2、6、12、14、16位为2'-氟代修饰；其余位置为2'-甲氧基修饰。硫代磷酸二酯基位于5'端第1和第2核苷酸、第2和第3核苷酸之间；3'端第1和第2核苷酸、第2和第3个苷酸之间。
ttcctggatcccgacagccgg

SEQ ID NO: 251 - RNA, 21 nt, synthetic construct
  source 1..21: mol_type = other RNA; note; note (original language) = 5'端带有乙烯基磷酸二酯基。第2、6、12、14、16位为2'-氟代修饰；其余位置为2'-甲氧基修饰。硫代磷酸二酯基位于5'端第1和第2核苷酸、第2和第3核苷酸之间；3'端第1和第2核苷酸、第2和第3个苷酸之间。
ttaggcaccaggggcttccca

SEQ ID NO: 252 - RNA, 21 nt, synthetic construct
  source 1..21: mol_type = other RNA; note; note (original language) = 5'端带有乙烯基磷酸二酯基。第2、6、12、14、16位为2'-氟代修饰；其余位置为2'-甲氧基修饰。硫代磷酸二酯基位于5'端第1和第2核苷酸、第2和第3核苷酸之间；3'端第1和第2核苷酸、第2和第3个苷酸之间。
ttggacctcctccagaggcac

SEQ ID NO: 253 - RNA, 21 nt, synthetic construct
  source 1..21: mol_type = other RNA; note; note (original language) = 5'端带有乙烯基磷酸二酯基。第2、6、12、14、16位为2'-氟代修饰；其余位置为2'-甲氧基修饰。硫代磷酸二酯基位于5'端第1和第2核苷酸、第2和第3核苷酸之间；3'端第1和第2核苷酸、第2和第3个苷酸之间。
tttgaggagagggctgggcag

SEQ ID NO: 254 - RNA, 21 nt, synthetic construct
  source 1..21: mol_type = other RNA; note; note (original language) = 5'端带有乙烯基磷酸二酯基。第2、6、12、14、16位为2'-氟代修饰；其余位置为2'-甲氧基修饰。硫代磷酸二酯基位于5'端第1和第2核苷酸、第2和第3核苷酸之间；3'端第1和第2核苷酸、第2和第3个苷酸之间。
tgcacgctcctcctcttcctc

SEQ ID NO: 255 - RNA, 21 nt, synthetic construct
  source 1..21: mol_type = other RNA; note; note (original language) = 5'端带有乙烯基磷酸二酯基。第2、6、12、14、16位为2'-氟代修饰；其余位置为2'-甲氧基修饰。硫代磷酸二酯基位于5'端第1和第2核苷酸、第2和第3核苷酸之间；3'端第1和第2核苷酸、第2和第3个苷酸之间。
ttgtggggggctctggttgta

SEQ ID NO: 256 - RNA, 21 nt, synthetic construct
  source 1..21: mol_type = other RNA; note; note (original language) = 5'端带有乙烯基磷酸二酯基。第2、6、12、14、16位为2'-氟代修饰；其余位置为2'-甲氧基修饰。硫代磷酸二酯基位于5'端第1和第2核苷酸、第2和第3核苷酸之间；3'端第1和第2核苷酸、第2和第3个苷酸之间。
tcattgtggggggctctggtt

SEQ ID NO: 257 - RNA, 21 nt, synthetic construct
  source 1..21: mol_type = other RNA; note; note (original language) = 5'端带有乙烯基磷酸二酯基。第2、6、12、14、16位为2'-氟代修饰；其余位置为2'-甲氧基修饰。硫代磷酸二酯基位于5'端第1和第2核苷酸、第2和第3核苷酸之间；3'端第1和第2核苷酸、第2和第3个苷酸之间。
tcgagccacactgtcccaggg

SEQ ID NO: 258 - RNA, 21 nt, synthetic construct
  source 1..21: mol_type = other RNA; note; note (original language) = 5'端带有乙烯基磷酸二酯基。第2、6、12、14、16位为2'-氟代修饰；其余位置为2'-甲氧基修饰。硫代磷酸二酯基位于5'端第1和第2核苷酸、第2和第3核苷酸之间；3'端第1和第2核苷酸、第2和第3个苷酸之间。
tggactcggtagttggacttg

SEQ ID NO: 259 - RNA, 21 nt, synthetic construct
  source 1..21: mol_type = other RNA; note; note (original language) = 5'端带有乙烯基磷酸二酯基。第2、6、12、14、16位为2'-氟代修饰；其余位置为2'-甲氧基修饰。硫代磷酸二酯基位于5'端第1和第2核苷酸、第2和第3核苷酸之间；3'端第1和第2核苷酸、第2和第3个苷酸之间。
tcggactcggtagttggactt

SEQ ID NO: 260 - RNA, 21 nt, synthetic construct
  source 1..21: mol_type = other RNA; note; note (original language) = 5'端带有乙烯基磷酸二酯基。第2、6、12、14、16位为2'-氟代修饰；其余位置为2'-甲氧基修饰。硫代磷酸二酯基位于5'端第1和第2核苷酸、第2和第3核苷酸之间；3'端第1和第2核苷酸、第2和第3个苷酸之间。
tccaatccgggctgtgatgtt

SEQ ID NO: 261 - RNA, 21 nt, synthetic construct
  source 1..21: mol_type = other RNA; note; note (original language) = 5'端带有乙烯基磷酸二酯基。第2、6、12、14、16位为2'-氟代修饰；其余位置为2'-甲氧基修饰。硫代磷酸二酯基位于5'端第1和第2核苷酸、第2和第3核苷酸之间；3'端第1和第2核苷酸、第2和第3个苷酸之间。
tcacacatgtccccaccttat

SEQ ID NO: 262 - RNA, 21 nt, synthetic construct
  source 1..21: mol_type = other RNA; note; note (original language) = 5'端带有乙烯基磷酸二酯基。第2、6、12、14、16位为2'-氟代修饰；其余位置为2'-甲氧基修饰。硫代磷酸二酯基位于5'端第1和第2核苷酸、第2和第3核苷酸之间；3'端第1和第2核苷酸、第2和第3个苷酸之间。
tacacacatgtccccacctta

SEQ ID NO: 263 - RNA, 21 nt, synthetic construct
  source 1..21: mol_type = other RNA; note; note (original language) = 5'端带有乙烯基磷酸二酯基。第2、6、12、14、16位为2'-氟代修饰；其余位置为2'-甲氧基修饰。硫代磷酸二酯基位于5'端第1和第2核苷酸、第2和第3核苷酸之间；3'端第1和第2核苷酸、第2和第3个苷酸之间。
tgacacacatgtccccacctt

SEQ ID NO: 264 - RNA, 21 nt, synthetic construct
  source 1..21: mol_type = other RNA; note; note (original language) = 5'端带有乙烯基磷酸二酯基。第2、6、12、14、16位为2'-氟代修饰；其余位置为2'-甲氧基修饰。硫代磷酸二酯基位于5'端第1和第2核苷酸、第2和第3核苷酸之间；3'端第1和第2核苷酸、第2和第3个苷酸之间。
tccctgcagggtagcttccct

SEQ ID NO: 265 - RNA, 21 nt, synthetic construct
  source 1..21: mol_type = other RNA; note; note (original language) = 5'端带有乙烯基磷酸二酯基。第2、6、12、14、16位为2'-氟代修饰；其余位置为2'-甲氧基修饰。硫代磷酸二酯基位于5'端第1和第2核苷酸、第2和第3核苷酸之间；3'端第1和第2核苷酸、第2和第3个苷酸之间。
ttccctgcagggtagcttccc

SEQ ID NO: 266 - RNA, 21 nt, synthetic construct
  source 1..21: mol_type = other RNA; note; note (original language) = 5'端带有乙烯基磷酸二酯基。第2、6、12、14、16位为2'-氟代修饰；其余位置为2'-甲氧基修饰。硫代磷酸二酯基位于5'端第1和第2核苷酸、第2和第3核苷酸之间；3'端第1和第2核苷酸、第2和第3个苷酸之间。
tgtccctgcagggtagcttcc

SEQ ID NO: 267 - RNA, 21 nt, synthetic construct
  source 1..21: mol_type = other RNA; note; note (original language) = 5'端带有乙烯基磷酸二酯基。第2、6、12、14、16位为2'-氟代修饰；其余位置为2'-甲氧基修饰。硫代磷酸二酯基位于5'端第1和第2核苷酸、第2和第3核苷酸之间；3'端第1和第2核苷酸、第2和第3个苷酸之间。
tctcagggtgtctcctggtct

SEQ ID NO: 268 - RNA, 21 nt, synthetic construct
  source 1..21: mol_type = other RNA; note; note (original language) = 5'端带有乙烯基磷酸二酯基。第2、6、12、14、16位为2'-氟代修饰；其余位置为2'-甲氧基修饰。硫代磷酸二酯基位于5'端第1和第2核苷酸、第2和第3核苷酸之间；3'端第1和第2核苷酸、第2和第3个苷酸之间。
ttctcagggtgtctcctggtc

SEQ ID NO: 269 - RNA, 19 nt, synthetic construct
  source 1..19: mol_type = other RNA; note; note (original language) = 第7-9位为2'-氟代修饰；其余位置为2'-甲氧基修饰。硫代磷酸二酯基位于5'端第1和第2核苷酸、第2和第3核苷酸之间；3'端第1和第2核苷酸、第2和第3个苷酸之间。5'端带有I-13'配体。
ctgtcagcatcagcatcaa

SEQ ID NO: 270 - RNA, 19 nt, synthetic construct
  source 1..19: mol_type = other RNA; note; note (original language) = 第7-9位为2'-氟代修饰；其余位置为2'-甲氧基修饰。硫代磷酸二酯基位于5'端第1和第2核苷酸、第2和第3核苷酸之间；3'端第1和第2核苷酸、第2和第3个苷酸之间。5'端带有I-13'配体。
gaccaactctctcctgtaa

SEQ ID NO: 271 - RNA, 19 nt, synthetic construct
  source 1..19: mol_type = other RNA; note; note (original language) = 第7-9位为2'-氟代修饰；其余位置为2'-甲氧基修饰。硫代磷酸二酯基位于5'端第1和第2核苷酸、第2和第3核苷酸之间；3'端第1和第2核苷酸、第2和第3个苷酸之间。5'端带有I-13'配体。
agaggaggagcgtgcagaa

SEQ ID NO: 272 - RNA, 19 nt, synthetic construct
  source 1..19: mol_type = other RNA; note; note (original language) = 第7-9位为2'-氟代修饰；其余位置为2'-甲氧基修饰。硫代磷酸二酯基位于5'端第1和第2核苷酸、第2和第3核苷酸之间；3'端第1和第2核苷酸、第2和第3个苷酸之间。5'端带有I-13'配体。
cagtcggagctaatggtga

SEQ ID NO: 273 - RNA, 19 nt, synthetic construct
  source 1..19: mol_type = other RNA; note; note (original language) = 第7-9位为2'-氟代修饰；其余位置为2'-甲氧基修饰。硫代磷酸二酯基位于5'端第1和第2核苷酸、第2和第3核苷酸之间；3'端第1和第2核苷酸、第2和第3个苷酸之间。5'端带有I-13'配体。
cttttctttttcccttgaa

SEQ ID NO: 274 - RNA, 19 nt, synthetic construct
  source 1..19: mol_type = other RNA; note; note (original language) = 第7-9位为2'-氟代修饰；其余位置为2'-甲氧基修饰。硫代磷酸二酯基位于5'端第1和第2核苷酸、第2和第3核苷酸之间；3'端第1和第2核苷酸、第2和第3个苷酸之间。5'端带有I-13'配体。
ccttttctttttcccttga

SEQ ID NO: 275 - RNA, 19 nt, Homo sapiens
  source 1..19: mol_type = mRNA
cgtgctgtcagcatcagca

SEQ ID NO: 276 - RNA, 21 nt, Homo sapiens
  source 1..21: mol_type = mRNA
tgctgatgctgacagcacggc

SEQ ID NO: 277 - RNA, 19 nt, Homo sapiens
  source 1..19: mol_type = mRNA
tgtcagcatcagcatcatc

SEQ ID NO: 278 - RNA, 21 nt, Homo sapiens
  source 1..21: mol_type = mRNA
gatgatgctgatgctgacagc